European Patent Application EP 4 516 320 A1, published March 5, 2025. Title: 一种包含亲水性糖结构的配体-药物偶联物. Applicant: 成都百利多特生物药业有限责任公司. The sequence listing filed with the application follows.

SEQUENCE LISTING (4 sequences)

SEQ ID NO: 1 - protein, 213 aa, synthetic construct
DIQMTQSPSSLSASVGDRVTITCRASQDINKYLAWYQQKPGKVPKLLIYSTSTLQSGVPSRFSGSGSGTDFTLTISSLQPEDVATYYCLQYDDLFTFGQGTKLEIKRTVAAPSVFIFPPSDEQLKSGTASVVCLLNNFYPREAKVQWKVDNALQSGNSQESVTEQDSKDSTYSLSSTLTLSKADYEKHKVYACEVTHQGLSSPVTKSFNRGEC

SEQ ID NO: 2 - protein, 447 aa, synthetic construct
QVQLVQSGAEVKKPGASVKLSCKASGYTFTSFDINWVRQAPEQRLEWMGWIFPGDGNTKYSQKFQGRATITRDTSASTAYMELSSLRSEDTAVYYCVRGEALYYFDYWGQGTLVTVSSASTKGPSVFPLAPSSKSTSGGTAALGCLVKDYFPEPVTVSWNSGALTSGVHTFPAVLQSSGLYSLSSVVTVPSSSLGTQTYICNVNHKPSNTKVDKRVEPKSCDKTHTCPPCPAPELLGGPSVFLFPPKPKDTLMISRTPEVTCVVVDVSHEDPEVKFNWYVDGVEVHNAKTKPREEQYNSTYRVVSVLTVLHQDWLNGKEYKCKVSNKALPAPIEKTISKAKGQPREPQVYTLPPSRDELTKNQVSLTCLVKGFYPSDIAVEWESNGQPENNYKTTPPVLDSDGSFFLYSKLTVDKSRWQQGNVFSCSVMHEALHNHYTQKSLSLSPG

SEQ ID NO: 3 - protein, 219 aa, synthetic construct
DIQLTQSPSTLSASVGDRVTITCRASESLDNYGIRFLTWFQQKPGKAPKLLMYAASNQGSGVPSRFSGSGSGTEFTLTISSLQPDDFATYYCQQTKEVPWSFGQGTKVEVKRTVAAPSVFIFPPSDEQLKSGTASVVCLLNNFYPREAKVQWKVDNALQSGNSQESVTEQDSKDSTYSLSSTLTLSKADYEKHKVYACEVTHQGLSSPVCTKSFNRGEC

SEQ ID NO: 4 - protein, 445 aa, synthetic construct
EVQLVQSGAEVKKPGSSVKVSCKASGYTITDSNIHWVRQAPGQSLEWIGYIYPYNGGTDYNQKFKNRATLTVDNPTNTAYMELSSLRSEDTAFYYCVNGNPWLAYWGQGTLVTVSSASTKGPSVFPLAPSSKSTSGGTAALGCLVKDYFPEPVTVSWNSGALTSGVHTFPAVLQSSGLYSLSSVVTVPSSSLGTQTYICNVNHKPSNTKVDKRVEPKSCDKTHTCPPCPAPELLGGPSVFLFPPKPKDTLMISRTPEVTCVVVDVSHEDPEVKFNWYVDGVEVHNAKTKPREEQYNSTYRVVSVLTVLHQDWLNGKEYKCKVSNKALPAPIEKTISKAKGQPREPQVYTLPPSRDELTKNQVSLTCLVKGFYPSDIAVEWESNGQPENNYKTTPPVLDSDGSFFLYSKLTVDKSRWQQGNVFSCSVMHEALHNHYTQKSLSLSPG